European Patent Specification EP 3 694 603 B1, published April 8, 2026. Title: Esophageal Tissue and/or Organoid Compositions and Methods of Making Same. Applicant: Children's Hosptial Medical Research Foundation. The sequence listing filed with the application follows.

SEQUENCE LISTING (82 sequences)

SEQ ID NO: 1 - DNA, 20 bp, Artificial Sequence
  DSG3 human forward primer
cgtggttgtctccgctagaa

SEQ ID NO: 2 - DNA, 20 bp, Artificial Sequence
  DSG3 human reverse primer
ccgaggtagcattgagggtt

SEQ ID NO: 3 - DNA, 20 bp, Artificial Sequence
  KRT5 human forward primer
ctggtccaactccttctcca

SEQ ID NO: 4 - DNA, 20 bp, Artificial Sequence
  KRT5 human reverse primer
ggagctcatgaacaccaagc

SEQ ID NO: 5 - DNA, 20 bp, Artificial Sequence
  FOXE1 human forward primer
cgacaaccccaaaaagtggc

SEQ ID NO: 6 - DNA, 20 bp, Artificial Sequence
  FOXE1 human reverse primer
gcccagtagttgcccttacc

SEQ ID NO: 7 - DNA, 20 bp, Artificial Sequence
  TBX1 human forward primer
gtctatgtggacccacgcaa

SEQ ID NO: 8 - DNA, 20 bp, Artificial Sequence
  TBX1 human reverse primer
ctgcgtgatccgatggttct

SEQ ID NO: 9 - DNA, 19 bp, Artificial Sequence
  SFRP2 human forward primer
ccaccgaggaagctccaaa

SEQ ID NO: 10 - DNA, 20 bp, Artificial Sequence
  SFRP2 human reverse primer
ttcaggtccctttcggacac

SEQ ID NO: 11 - DNA, 20 bp, Artificial Sequence
  SOX2 human forward primer
gcttagcctcgtcgatgaac

SEQ ID NO: 12 - DNA, 20 bp, Artificial Sequence
  SOX2 human reverse primer
aaccccaagatgcacaactc

SEQ ID NO: 13 - DNA, 20 bp, Artificial Sequence
  PAX9 human forward primer
ggtagggtaaggagccatgc

SEQ ID NO: 14 - DNA, 20 bp, Artificial Sequence
  PAX9 human reverse primer
ctggagcaggaagccaagta

SEQ ID NO: 15 - DNA, 20 bp, Artificial Sequence
  GATA4 human forward primer
tagccccacagttgacacac

SEQ ID NO: 16 - DNA, 17 bp, Artificial Sequence
  GATA4 human reverse primer
gtcctgcacagcctgcc

SEQ ID NO: 17 - DNA, 20 bp, Artificial Sequence
  KRT13 human forward primer
aggtgaagatccgtgactgg

SEQ ID NO: 18 - DNA, 19 bp, Artificial Sequence
  KRT13 human reverse primer
gttgttttcaatggtggcg

SEQ ID NO: 19 - DNA, 20 bp, Artificial Sequence
  KRT14 human forward primer
ggcctgctgagatcaaagac

SEQ ID NO: 20 - DNA, 19 bp, Artificial Sequence
  KRT14 human reverse primer
tctgcagaaggacattggc

SEQ ID NO: 21 - DNA, 20 bp, Artificial Sequence
  IVL human forward primer
ctgcctcagccttactgtga

SEQ ID NO: 22 - DNA, 21 bp, Artificial Sequence
  IVL human reverse primer
ggaggaggaacagtcttgagg

SEQ ID NO: 23 - DNA, 20 bp, Artificial Sequence
  LEF1 human forward primer
cactgtaagtgatgaggggg

SEQ ID NO: 24 - DNA, 20 bp, Artificial Sequence
  LEF1 human reverse primer
tggatctctttctccaccca

SEQ ID NO: 25 - DNA, 20 bp, Artificial Sequence
  TCF1 human forward primer
gacttgaccatcttcgccac

SEQ ID NO: 26 - DNA, 21 bp, Artificial Sequence
  TCF1 human reverse primer
cctcaaagagctggagaacct

SEQ ID NO: 27 - DNA, 23 bp, Artificial Sequence
  HNF1B human forward primer
tcacagataccagcagcatcagt

SEQ ID NO: 28 - DNA, 19 bp, Artificial Sequence
  HNF1B human reverse primer
gggcatcaccaggcttgta

SEQ ID NO: 29 - DNA, 20 bp, Artificial Sequence
  PROX1 human forward primer
ggcattgaaaaactcccgta

SEQ ID NO: 30 - DNA, 20 bp, Artificial Sequence
  PROX1 human reverse primer
acagggctctgaacatgcac

SEQ ID NO: 31 - DNA, 20 bp, Artificial Sequence
  HNF6 human forward primer
tgttgcctctatccttccca

SEQ ID NO: 32 - DNA, 19 bp, Artificial Sequence
  HNF6 human reverse primer
ggaggatgtggaagtggct

SEQ ID NO: 33 - DNA, 18 bp, Artificial Sequence
  PDX1 human forward primer
cgtccgcttgttctcctc

SEQ ID NO: 34 - DNA, 20 bp, Artificial Sequence
  PDX1 human reverse primer
cctttcccatggatgaagtc

SEQ ID NO: 35 - DNA, 20 bp, Artificial Sequence
  DeltaN isoform human forward primer
agccagaagaaaggacagca

SEQ ID NO: 36 - DNA, 21 bp, Artificial Sequence
  DeltaN isoform human reverse primer
tcgtgtactgtggctcactaa

SEQ ID NO: 37 - DNA, 21 bp, Artificial Sequence
  RFX6 human forward primer
ccagtttttgagctaagcgaa

SEQ ID NO: 38 - DNA, 20 bp, Artificial Sequence
  RFX6 human reverse primer
tggcatcaaagagagcagtg

SEQ ID NO: 39 - DNA, 19 bp, Artificial Sequence
  MNX1 human forward primer
ctgcctaagatgcccgact

SEQ ID NO: 40 - DNA, 18 bp, Artificial Sequence
  MNX1 human reverse primer
agctgctggctggtgaag

SEQ ID NO: 41 - DNA, 18 bp, Artificial Sequence
  NKX2-1 (TTF1) human forward primer
ctcatgttcatgccgctc

SEQ ID NO: 42 - DNA, 19 bp, Artificial Sequence
  NKX2-1 (TTF1) human reverse primer
gacaccatgaggaacagcg

SEQ ID NO: 43 - DNA, 19 bp, Artificial Sequence
  CDH1 (E-CAD) human forward primer
gaccggtgcaatcttcaaa

SEQ ID NO: 44 - DNA, 19 bp, Artificial Sequence
  CDH1 (E-CAD) human reverse primer
ttgacgccgagagctacac

SEQ ID NO: 45 - DNA, 20 bp, Artificial Sequence
  AXIN2 human forward primer
ctggtgcaaagacatagcca

SEQ ID NO: 46 - DNA, 20 bp, Artificial Sequence
  AXIN2 human reverse primer
agtgtgaggtccacggaaac

SEQ ID NO: 47 - DNA, 20 bp, Artificial Sequence
  KRT4 human forward primer
cctgagatccagaaagtccg

SEQ ID NO: 48 - DNA, 20 bp, Artificial Sequence
  KRT4 human reverse primer
ttccatttggtctccaggac

SEQ ID NO: 49 - DNA, 22 bp, Artificial Sequence
  CDX2 human forward primer
ctggagctggagaaggagtttc

SEQ ID NO: 50 - DNA, 24 bp, Artificial Sequence
  CDX2 human reverse primer
attttaacctgcctctcagagagc

SEQ ID NO: 51 - DNA, 20 bp, Artificial Sequence
  NESTIN human forward primer
gagggaagtcttggagccac

SEQ ID NO: 52 - DNA, 19 bp, Artificial Sequence
  NESTIN human reverse primer
aagatgtccctcagcctgg

SEQ ID NO: 53 - DNA, 20 bp, Artificial Sequence
  HOXA1 human forward primer
gtacggctacctgggtcaac

SEQ ID NO: 54 - DNA, 20 bp, Artificial Sequence
  HOXA1 human reverse primer
acttgggtctcgttgagctg

SEQ ID NO: 55 - DNA, 20 bp, Artificial Sequence
  HOXB1 human forward primer
aacccacccaagacagcgaa

SEQ ID NO: 56 - DNA, 21 bp, Artificial Sequence
  HOXB1 human reverse primer
cgcgcttcttctgcttcattc

SEQ ID NO: 57 - DNA, 20 bp, Artificial Sequence
  CYP26C1 human forward primer
gttcccttcagtggcctacg

SEQ ID NO: 58 - DNA, 20 bp, Artificial Sequence
  CYP26C1 human reverse primer
acagccgactccttcagctc

SEQ ID NO: 59 - DNA, 22 bp, Artificial Sequence
  OTX2 human forward primer
ggaagcactgtttgccaagacc

SEQ ID NO: 60 - DNA, 22 bp, Artificial Sequence
  OTX2 human reverse primer
ctgttgttggcggcacttagct

SEQ ID NO: 61 - DNA, 21 bp, Artificial Sequence
  CRNN human forward primer
tgtgattgtgaaaccccacga

SEQ ID NO: 62 - DNA, 20 bp, Artificial Sequence
  CRNN human reverse primer
gcactctcgctcagtgtctt

SEQ ID NO: 63 - DNA, 22 bp, Artificial Sequence
  TMPRSS11A human forward primer
gtctcctggttcacttcctagt

SEQ ID NO: 64 - DNA, 22 bp, Artificial Sequence
  TMPRSS11A human reverse primer
gtgttgctttgtccgaaattgt

SEQ ID NO: 65 - DNA, 22 bp, Artificial Sequence
  TMPRSS11D human forward primer
gcagtcaccatagctctacttg

SEQ ID NO: 66 - DNA, 23 bp, Artificial Sequence
  TMPRSS11D human reverse primer
ccactcaaagtcctgtattcctg

SEQ ID NO: 67 - DNA, 21 bp, Artificial Sequence
  CPHA (PPIA) human forward primer
cccaccgtgttcttcgacatt

SEQ ID NO: 68 - DNA, 22 bp, Artificial Sequence
  CPHA (PPIA) human reverse primer
ggacccgtatgctttaggatga

SEQ ID NO: 69 - DNA, 20 bp, Artificial Sequence
  ID1 human forward primer
ctgctctacgacatgaacgg

SEQ ID NO: 70 - DNA, 22 bp, Artificial Sequence
  ID1 human reverse primer
gaaggtccctgatgtagtcgat

SEQ ID NO: 71 - DNA, 20 bp, Artificial Sequence
  ID3 human forward primer
gagaggcactcagcttagcc

SEQ ID NO: 72 - DNA, 22 bp, Artificial Sequence
  ID3 human reverse primer
tccttttgtcgttggagatgac

SEQ ID NO: 73 - DNA, 20 bp, Artificial Sequence
  HES5 human forward primer
gaaaaaccgactgcggaagc

SEQ ID NO: 74 - DNA, 20 bp, Artificial Sequence
  HES5 human reverse primer
gacgaaggctttgctgtgct

SEQ ID NO: 75 - DNA, 20 bp, Artificial Sequence
  FST human forward primer
tgccacctgagaaaggctac

SEQ ID NO: 76 - DNA, 25 bp, Artificial Sequence
  FST human reverse primer
tcttcacaggactttgctttgatac

SEQ ID NO: 77 - DNA, 20 bp, Artificial Sequence
  NOG human forward primer
tggtggacctcatcgaacac

SEQ ID NO: 78 - DNA, 20 bp, Artificial Sequence
  NOG human reverse primer
atgaagcctgggtcgtagtg

SEQ ID NO: 79 - DNA, 27 bp, Artificial Sequence
  CCL26 human forward primer
aactccgaaacaattgtgactcagctg

SEQ ID NO: 80 - DNA, 24 bp, Artificial Sequence
  CCL26 human reverse primer
gtaactctgggaggaaacaccctc

SEQ ID NO: 81 - DNA, 21 bp, Artificial Sequence
  CDH26 human forward primer
tgctttttctgttgcgatgct

SEQ ID NO: 82 - DNA, 19 bp, Artificial Sequence
  CDH26 human reverse primer
cttgccataaccccagctc